European Patent Application EP 4 397 765 A2, published July 10, 2024. Title: METHOD FOR CHANGING THE INTERCELLULAR MOBILITY OF AN MRNA. Applicant: Rijk Zwaan Zaadteelt en Zaadhandel B.V. Application EP EP23177043.9, filed April 13, 2017. The sequence listing filed with the application follows.

SEQUENCE LISTING (110 sequences)

SEQ ID NO: 1 - DNA, 20 bp, Nicotiana tabacum
  misc_feature 1..20: note = source = /organism="Nicotiana tabacum" /note="Table 2: FK868-F" /mol_type="unassigned DNA"
  source 1..20: mol_type = genomic DNA
gatgctccgaatctcgctga

SEQ ID NO: 2 - DNA, 20 bp, Nicotiana tabacum
  misc_feature 1..20: note = source = /organism="Nicotiana tabacum" /note="Table 2: FK869-R" /mol_type="unassigned DNA"
  source 1..20: mol_type = genomic DNA
gttgcttgctgctggtgaag

SEQ ID NO: 3 - DNA, 20 bp, Nicotiana tabacum
  misc_feature 1..20: note = source = /organism="Nicotiana tabacum" /note="Table 2: FK868-F" /mol_type="unassigned DNA"
  source 1..20: mol_type = genomic DNA
gatgctccgaatctcgctga

SEQ ID NO: 4 - DNA, 21 bp, Nicotiana tabacum
  misc_feature 1..21: note = source = /organism="Nicotiana tabacum" /note="Table 2: FK851-R" /mol_type="unassigned DNA"
  source 1..21: mol_type = genomic DNA
ttccgctgcgccactctgatt

SEQ ID NO: 5 - DNA, 20 bp, Nicotiana tabacum
  misc_feature 1..20: note = source = /organism="Nicotiana tabacum" /note="Table 2: FK868-F" /mol_type="unassigned DNA"
  source 1..20: mol_type = genomic DNA
gatgctccgaatctcgctga

SEQ ID NO: 6 - DNA, 21 bp, Nicotiana tabacum
  misc_feature 1..21: note = source = /organism="Nicotiana tabacum" /note="Table 2: FK851-R" /mol_type="unassigned DNA"
  source 1..21: mol_type = genomic DNA
ttccgctgcgccactctgatt

SEQ ID NO: 7 - DNA, 20 bp, Nicotiana tabacum
  misc_feature 1..20: note = source = /organism="Nicotiana tabacum" /note="Table 2: FK868-F" /mol_type="unassigned DNA"
  source 1..20: mol_type = genomic DNA
gatgctccgaatctcgctga

SEQ ID NO: 8 - DNA, 18 bp, Nicotiana tabacum
  misc_feature 1..18: note = source = /organism="Nicotiana tabacum" /note="Table 2: FK779-R" /mol_type="unassigned DNA"
  source 1..18: mol_type = genomic DNA
tagaaggcattggtggtg

SEQ ID NO: 9 - DNA, 18 bp, Nicotiana tabacum
  misc_feature 1..18: note = source = /organism="Nicotiana tabacum" /note="Table 2: FK774-F" /mol_type="unassigned DNA"
  source 1..18: mol_type = genomic DNA
ataacccacaggtcccag

SEQ ID NO: 10 - DNA, 18 bp, Nicotiana tabacum
  misc_feature 1..18: note = source = /organism="Nicotiana tabacum" /note="Table 2: FK771-R" /mol_type="unassigned DNA"
  source 1..18: mol_type = genomic DNA
ttccattccctcctttca

SEQ ID NO: 11 - DNA, 20 bp, Nicotiana tabacum
  misc_feature 1..20: note = source = /organism="Nicotiana tabacum" /note="Table 2: FK938-F" /mol_type="unassigned DNA"
  source 1..20: mol_type = genomic DNA
cccgacaaccactacctgag

SEQ ID NO: 12 - DNA, 23 bp, Nicotiana tabacum
  misc_feature 1..23: note = source = /organism="Nicotiana tabacum" /note="Table 2: FK858-R" /mol_type="unassigned DNA"
  source 1..23: mol_type = genomic DNA
tcatcgagagcttgacaccctgt

SEQ ID NO: 13 - DNA, 21 bp, Nicotiana tabacum
  misc_feature 1..21: note = source = /organism="Nicotiana tabacum" /note="Table 2: FK422-F" /mol_type="unassigned DNA"
  source 1..21: mol_type = genomic DNA
caccggtattgtgttggactc

SEQ ID NO: 14 - DNA, 23 bp, Nicotiana tabacum
  misc_feature 1..23: note = source = /organism="Nicotiana tabacum" /note="Table 2: FK423-R" /mol_type="unassigned DNA"
  source 1..23: mol_type = genomic DNA
aggacctcaggacaacggaaacg

SEQ ID NO: 15 - DNA, 20 bp, Nicotiana tabacum
  misc_feature 1..20: note = source = /organism="Nicotiana tabacum" /note="Table 2: FK424-F" /mol_type="unassigned DNA"
  source 1..20: mol_type = genomic DNA
ggaaggatctgtacggtaac

SEQ ID NO: 16 - DNA, 20 bp, Nicotiana tabacum
  misc_feature 1..20: note = source = /organism="Nicotiana tabacum" /note="Table 2: FK425-R" /mol_type="unassigned DNA"
  source 1..20: mol_type = genomic DNA
tgtgaacgattcctggacct

SEQ ID NO: 17 - DNA, 19 bp, Nicotiana tabacum
  misc_feature 1..19: note = source = /organism="Nicotiana tabacum" /note="Table 2: FK907-F" /mol_type="unassigned DNA"
  source 1..19: mol_type = genomic DNA
attttgccgatttcggaac

SEQ ID NO: 18 - DNA, 21 bp, Nicotiana tabacum
  misc_feature 1..21: note = source = /organism="Nicotiana tabacum" /note="Table 2: FK908-R" /mol_type="unassigned DNA"
  source 1..21: mol_type = genomic DNA
tggttcattacaggagaaccg

SEQ ID NO: 19 - DNA, 21 bp, Nicotiana tabacum
  misc_feature 1..21: note = source = /organism="Nicotiana tabacum" /note="Table 2: FK909-F" /mol_type="unassigned DNA"
  source 1..21: mol_type = genomic DNA
tttgtgaatctcagggaatgc

SEQ ID NO: 20 - DNA, 21 bp, Nicotiana tabacum
  misc_feature 1..21: note = source = /organism="Nicotiana tabacum" /note="Table 2: FK914-R" /mol_type="unassigned DNA"
  source 1..21: mol_type = genomic DNA
agcagccatctcacaaaagtg

SEQ ID NO: 21 - DNA, 21 bp, Nicotiana tabacum
  misc_feature 1..21: note = source = /organism="Nicotiana tabacum" /note="Table 2: FK915-R" /mol_type="unassigned DNA"
  source 1..21: mol_type = genomic DNA
tctaaaacgcgttttgcaaac

SEQ ID NO: 22 - DNA, 20 bp, Nicotiana tabacum
  misc_feature 1..20: note = source = /organism="Nicotiana tabacum" /note="Table 2: FK883-F" /mol_type="unassigned DNA"
  source 1..20: mol_type = genomic DNA
ctatggggaatcatctcggg

SEQ ID NO: 23 - DNA, 20 bp, Nicotiana tabacum
  misc_feature 1..20: note = source = /organism="Nicotiana tabacum" /note="Table 2: FK884-R" /mol_type="unassigned DNA"
  source 1..20: mol_type = genomic DNA
cactagaccactggtgcttc

SEQ ID NO: 24 - DNA, 20 bp, Nicotiana tabacum
  misc_feature 1..20: note = source = /organism="Nicotiana tabacum" /note="Table 2: FK883-F" /mol_type="unassigned DNA"
  source 1..20: mol_type = genomic DNA
ctatggggaatcatctcggg

SEQ ID NO: 25 - DNA, 20 bp, Nicotiana tabacum
  misc_feature 1..20: note = source = /organism="Nicotiana tabacum" /note="Table 2: FK992-R" /mol_type="unassigned DNA"
  source 1..20: mol_type = genomic DNA
ccgtggcagggtactatcat

SEQ ID NO: 26 - DNA, 20 bp, Nicotiana tabacum
  misc_feature 1..20: note = source = /organism="Nicotiana tabacum" /note="Table 2: FK883-F" /mol_type="unassigned DNA"
  source 1..20: mol_type = genomic DNA
ctatggggaatcatctcggg

SEQ ID NO: 27 - DNA, 25 bp, Nicotiana tabacum
  misc_feature 1..25: note = source = /organism="Nicotiana tabacum" /note="Table 2: FK962-R" /mol_type="unassigned DNA"
  source 1..25: mol_type = genomic DNA
gtagactatatattgtggtgtaaac

SEQ ID NO: 28 - DNA, 21 bp, Nicotiana tabacum
  misc_feature 1..21: note = source = /organism="Nicotiana tabacum" /note="Table 2: FK963-F" /mol_type="unassigned DNA"
  source 1..21: mol_type = genomic DNA
ctagccatggtagatctgagg

SEQ ID NO: 29 - DNA, 106 bp, Nicotiana tabacum
  misc_feature 1..106: note = source = /organism="Nicotiana tabacum" /note="Table 2: FK944-R" /mol_type="unassigned DNA"
  source 1..106: mol_type = genomic DNA
gcgcggtgacctgcaccagccgggaattgaacccgggtctgtaccgtggcagggtactatcatgccactagaccactggtgcaattcacacgtgatggtgatggtg

SEQ ID NO: 30 - DNA, 106 bp, Nicotiana tabacum
  misc_feature 1..106: note = source = /organism="Nicotiana tabacum" /note="Table 2: FK945-R" /mol_type="unassigned DNA"
  source 1..106: mol_type = genomic DNA
gcgcggtgacctatcagagccaccttcgatcctgggacctgtgggttatgggcccaccacgcttccgctgcgccactctgataattcacacgtgatggtgatggtg

SEQ ID NO: 31 - DNA, 108 bp, Nicotiana tabacum
  misc_feature 1..108: note = source = /organism="Nicotiana tabacum" /note="Table 2: FK946-R" /mol_type="unassigned DNA"
  source 1..108: mol_type = genomic DNA
gcgcggtgaccgcttccggcggggctcgaacccgcgaccttcggctcataagaccaacgctctaaccaactgagctacgggagcaattcacacgtgatggtgatggtg

SEQ ID NO: 32 - DNA, 94 bp, Nicotiana tabacum
  misc_feature 1..94: note = source = /organism="Nicotiana tabacum" /note="Table 2: FK948-R" /mol_type="unassigned DNA"
  source 1..94: mol_type = genomic DNA
gcgcggtgacctatcagagccaggtttcgatcctgggacctgtgggttatgggcccaccaccactctgataattcacacgtgatggtgatggtg

SEQ ID NO: 33 - DNA, 79 bp, Nicotiana tabacum
  misc_feature 1..79: note = source = /organism="Nicotiana tabacum" /note="Table 2: FK950-R" /mol_type="unassigned DNA"
  source 1..79: mol_type = genomic DNA
gcgcggtgacctatcagagccaggtttcgatcctgggacctgccaccactctgataattcacacgtgatggtgatggtg

SEQ ID NO: 34 - DNA, 79 bp, Nicotiana tabacum
  misc_feature 1..79: note = source = /organism="Nicotiana tabacum" /note="Table 2: FK949-R" /mol_type="unassigned DNA"
  source 1..79: mol_type = genomic DNA
gcgcggtgacctatcagagcggacctgtgggttatgggcccaccaccactctgacaattcacacgtgatggtgatggtg

SEQ ID NO: 35 - DNA, 77 bp, Nicotiana tabacum
  misc_feature 1..77: note = source = /organism="Nicotiana tabacum" /note="Table 2: FK947-R" /mol_type="unassigned DNA"
  source 1..77: mol_type = genomic DNA
gcgcggtgacctatcagagcggacctgccacgcttccgctgcgccactctgataattcacacgtgatggtgatggtg

SEQ ID NO: 36 - DNA, 26 bp, Nicotiana tabacum
  misc_feature 1..26: note = source = /organism="Nicotiana tabacum" /note="Table 2: FK951-R" /mol_type="unassigned DNA"
  source 1..26: mol_type = genomic DNA
gcgcggtgacctctagatatcagagc

SEQ ID NO: 37 - DNA, 23 bp, Nicotiana tabacum
  misc_feature 1..23: note = source = /organism="Nicotiana tabacum" /note="Table 2: FK952-R" /mol_type="unassigned DNA"
  source 1..23: mol_type = genomic DNA
gcgcggtgacctctagatgcacc

SEQ ID NO: 38 - DNA, 25 bp, Nicotiana tabacum
  misc_feature 1..25: note = source = /organism="Nicotiana tabacum" /note="Table 2: FK953-R" /mol_type="unassigned DNA"
  source 1..25: mol_type = genomic DNA
gcgcggtgacctctagagcttccgg

SEQ ID NO: 39 - DNA, 20 bp, Nicotiana tabacum
  misc_feature 1..20: note = source = /organism="Nicotiana tabacum" /note="Table 2: FK1091-F" /mol_type="unassigned DNA"
  source 1..20: mol_type = genomic DNA
caacagcttccggaccgcac

SEQ ID NO: 40 - DNA, 20 bp, Nicotiana tabacum
  misc_feature 1..20: note = source = /organism="Nicotiana tabacum" /note="Table 2: FK1092-R" /mol_type="unassigned DNA"
  source 1..20: mol_type = genomic DNA
gattgagcgcgatgacgtca

SEQ ID NO: 41 - DNA, 20 bp, Nicotiana tabacum
  misc_feature 1..20: note = source = /organism="Nicotiana tabacum" /note="Table 2: FK1079-F" /mol_type="unassigned DNA"
  source 1..20: mol_type = genomic DNA
cgagtactaccaggcgaacc

SEQ ID NO: 42 - DNA, 21 bp, Nicotiana tabacum
  misc_feature 1..21: note = source = /organism="Nicotiana tabacum" /note="Table 2: FK1079-F" /mol_type="unassigned DNA"
  source 1..21: mol_type = genomic DNA
cagagccaggtttcgatcctg

SEQ ID NO: 43 - DNA, 20 bp, Nicotiana tabacum
  misc_feature 1..20: note = source = /organism="Nicotiana tabacum" /note="Table 2: FK1079-F" /mol_type="unassigned DNA"
  source 1..20: mol_type = genomic DNA
cgagtactaccaggcgaacc

SEQ ID NO: 44 - DNA, 20 bp, Nicotiana tabacum
  misc_feature 1..20: note = source = /organism="Nicotiana tabacum" /note="Table 2: FK1086-R" /mol_type="unassigned DNA"
  source 1..20: mol_type = genomic DNA
gcagggtactatcatgccac

SEQ ID NO: 45 - DNA, 20 bp, Nicotiana tabacum
  misc_feature 1..20: note = source = /organism="Nicotiana tabacum" /note="Table 2: FK1080-F" /mol_type="unassigned DNA"
  source 1..20: mol_type = genomic DNA
accacgtcgtgttcgatgag

SEQ ID NO: 46 - DNA, 20 bp, Nicotiana tabacum
  misc_feature 1..20: note = source = /organism="Nicotiana tabacum" /note="Table 2: FK1085-R" /mol_type="unassigned DNA"
  source 1..20: mol_type = genomic DNA
ggctcataagaccaacgctc

SEQ ID NO: 47 - DNA, 20 bp, Nicotiana tabacum
  misc_feature 1..20: note = source = /organism="Nicotiana tabacum" /note="Table 2: FK1079-F" /mol_type="unassigned DNA"
  source 1..20: mol_type = genomic DNA
cgagtactaccaggcgaacc

SEQ ID NO: 48 - DNA, 21 bp, Nicotiana tabacum
  misc_feature 1..21: note = source = /organism="Nicotiana tabacum" /note="Table 2: FK1081-R" /mol_type="unassigned DNA"
  source 1..21: mol_type = genomic DNA
cagagccaggtttcgatcctg

SEQ ID NO: 49 - DNA, 20 bp, Nicotiana tabacum
  misc_feature 1..20: note = source = /organism="Nicotiana tabacum" /note="Table 2: FK1080-F" /mol_type="unassigned DNA"
  source 1..20: mol_type = genomic DNA
accacgtcgtgttcgatgag

SEQ ID NO: 50 - DNA, 21 bp, Nicotiana tabacum
  misc_feature 1..21: note = source = /organism="Nicotiana tabacum" /note="Table 2: FK1083-R" /mol_type="unassigned DNA"
  source 1..21: mol_type = genomic DNA
gttatgggcccaccaccactc

SEQ ID NO: 51 - DNA, 20 bp, Nicotiana tabacum
  misc_feature 1..20: note = source = /organism="Nicotiana tabacum" /note="Table 2: FK1079-F" /mol_type="unassigned DNA"
  source 1..20: mol_type = genomic DNA
cgagtactaccaggcgaacc

SEQ ID NO: 52 - DNA, 18 bp, Nicotiana tabacum
  misc_feature 1..18: note = source = /organism="Nicotiana tabacum" /note="Table 2: FK1084-R" /mol_type="unassigned DNA"
  source 1..18: mol_type = genomic DNA
gatcctgggacctgccac

SEQ ID NO: 53 - DNA, 20 bp, Nicotiana tabacum
  misc_feature 1..20: note = source = /organism="Nicotiana tabacum" /note="Table 2: FK1079-F" /mol_type="unassigned DNA"
  source 1..20: mol_type = genomic DNA
cgagtactaccaggcgaacc

SEQ ID NO: 54 - DNA, 21 bp, Nicotiana tabacum
  misc_feature 1..21: note = source = /organism="Nicotiana tabacum" /note="Table 2: FK1082-R" /mol_type="unassigned DNA"
  source 1..21: mol_type = genomic DNA
gctgcgccactctgataattc

SEQ ID NO: 55 - DNA, 21 bp, Nicotiana tabacum
  misc_feature 1..21: note = source = /organism="Nicotiana tabacum" /note="Table 2: FK1099-F" /mol_type="unassigned DNA"
  source 1..21: mol_type = genomic DNA
agaacgctagccatcaccatc

SEQ ID NO: 56 - DNA, 22 bp, Nicotiana tabacum
  misc_feature 1..22: note = source = /organism="Nicotiana tabacum" /note="Table 2: FK1100-R" /mol_type="unassigned DNA"
  source 1..22: mol_type = genomic DNA
gccaaatgtttgaacgatcggg

SEQ ID NO: 57 - DNA, 21 bp, Nicotiana tabacum
  misc_feature 1..21: note = source = /organism="Nicotiana tabacum" /note="Table 2: FK1099-F" /mol_type="unassigned DNA"
  source 1..21: mol_type = genomic DNA
agaacgctagccatcaccatc

SEQ ID NO: 58 - DNA, 19 bp, Nicotiana tabacum
  misc_feature 1..19: note = source = /organism="Nicotiana tabacum" /note="Table 2: FK1090-R" /mol_type="unassigned DNA"
  source 1..19: mol_type = genomic DNA
gcaagaccggcaacaggat

SEQ ID NO: 59 - DNA, 21 bp, Nicotiana tabacum
  misc_feature 1..21: note = source = /organism="Nicotiana tabacum" /note="Table 2: FK1093-F" /mol_type="unassigned DNA"
  source 1..21: mol_type = genomic DNA
cgcgtccaaggaaacaagaag

SEQ ID NO: 60 - DNA, 23 bp, Nicotiana tabacum
  misc_feature 1..23: note = source = /organism="Nicotiana tabacum" /note="Table 2: FK1094-F" /mol_type="unassigned DNA"
  source 1..23: mol_type = genomic DNA
ttcacacgtgatggtgatggtga

SEQ ID NO: 61 - DNA, 23 bp, Nicotiana tabacum
  misc_feature 1..23: note = source = /organism="Nicotiana tabacum" /note="Table 2: FK1097-F" /mol_type="unassigned DNA"
  source 1..23: mol_type = genomic DNA
tccctcagcacattccagcagat

SEQ ID NO: 62 - DNA, 24 bp, Nicotiana tabacum
  misc_feature 1..24: note = source = /organism="Nicotiana tabacum" /note="Table 2: FK1098-F" /mol_type="unassigned DNA"
  source 1..24: mol_type = genomic DNA
aacgattcctggacctgcctcatc

SEQ ID NO: 63 - DNA, 22 bp, Nicotiana tabacum
  misc_feature 1..22: note = source = /organism="Nicotiana tabacum" /note="Table 2: FK1095-F" /mol_type="unassigned DNA"
  source 1..22: mol_type = genomic DNA
cacacttcacttggtcttgcgt

SEQ ID NO: 64 - DNA, 24 bp, Nicotiana tabacum
  misc_feature 1..24: note = source = /organism="Nicotiana tabacum" /note="Table 2: FK1096-R" /mol_type="unassigned DNA"
  source 1..24: mol_type = genomic DNA
tagtctttccggtgagagtcttca

SEQ ID NO: 65 - DNA, 21 bp, Nicotiana tabacum
  misc_feature 1..21: note = source = /organism="Nicotiana tabacum" /note="Table 2: FK1105-F" /mol_type="unassigned DNA"
  source 1..21: mol_type = genomic DNA
atcttctggggactatgggga

SEQ ID NO: 66 - DNA, 22 bp, Nicotiana tabacum
  misc_feature 1..22: note = source = /organism="Nicotiana tabacum" /note="Table 2: FK1106-R" /mol_type="unassigned DNA"
  source 1..22: mol_type = genomic DNA
tcatccttcaagaagcaaaggc

SEQ ID NO: 67 - DNA, 22 bp, Nicotiana tabacum
  misc_feature 1..22: note = source = /organism="Nicotiana tabacum" /note="Table 2: FK1107-F" /mol_type="unassigned DNA"
  source 1..22: mol_type = genomic DNA
tcatacacgccagaactctttc

SEQ ID NO: 68 - DNA, 24 bp, Nicotiana tabacum
  misc_feature 1..24: note = source = /organism="Nicotiana tabacum" /note="Table 2: FK1108-R" /mol_type="unassigned DNA"
  source 1..24: mol_type = genomic DNA
ccaaccgatacttatccatctcta

SEQ ID NO: 69 - DNA, 24 bp, Nicotiana tabacum
  misc_feature 1..24: note = source = /organism="Nicotiana tabacum" /note="Table 2: FK1122-F" /mol_type="unassigned DNA"
  source 1..24: mol_type = genomic DNA
ccggattcttcatcttctctctct

SEQ ID NO: 70 - DNA, 27 bp, Nicotiana tabacum
  misc_feature 1..27: note = source = /organism="Nicotiana tabacum" /note="Table 2: FK1123-R" /mol_type="unassigned DNA"
  source 1..27: mol_type = genomic DNA
cctaagcgagaatcataccactagacc

SEQ ID NO: 71 - DNA, 25 bp, Nicotiana tabacum
  misc_feature 1..25: note = source = /organism="Nicotiana tabacum" /note="Table 2: FK1124-F" /mol_type="unassigned DNA"
  source 1..25: mol_type = genomic DNA
gttacagtagcagagaggtcttaca

SEQ ID NO: 72 - DNA, 22 bp, Nicotiana tabacum
  misc_feature 1..22: note = source = /organism="Nicotiana tabacum" /note="Table 2: FK1125-R" /mol_type="unassigned DNA"
  source 1..22: mol_type = genomic DNA
cgagttcaattctcggaatgcc

SEQ ID NO: 73 - DNA, 24 bp, Nicotiana tabacum
  misc_feature 1..24: note = source = /organism="Nicotiana tabacum" /note="Table 2: FK1126-F" /mol_type="unassigned DNA"
  source 1..24: mol_type = genomic DNA
caacagaccaaactaagaaagctc

SEQ ID NO: 74 - DNA, 22 bp, Nicotiana tabacum
  misc_feature 1..22: note = source = /organism="Nicotiana tabacum" /note="Table 2: FK1125-R" /mol_type="unassigned DNA"
  source 1..22: mol_type = genomic DNA
cgagttcaattctcggaatgcc

SEQ ID NO: 75 - DNA, 27 bp, Nicotiana tabacum
  misc_feature 1..27: note = source = /organism="Nicotiana tabacum" /note="Table 2: FK1127-F" /mol_type="unassigned DNA"
  source 1..27: mol_type = genomic DNA
cctttagaagatactcgatttggtgtc

SEQ ID NO: 76 - DNA, 23 bp, Nicotiana tabacum
  misc_feature 1..23: note = source = /organism="Nicotiana tabacum" /note="Table 2: FK1128-R" /mol_type="unassigned DNA"
  source 1..23: mol_type = genomic DNA
gtctgattagaagtcagacgcct

SEQ ID NO: 77 - DNA, 20 bp, Nicotiana tabacum
  misc_feature 1..20: note = source = /organism="Nicotiana tabacum" /note="Table 2: FK1129-F" /mol_type="unassigned DNA"
  source 1..20: mol_type = genomic DNA
cgacataaaagcaccgttcc

SEQ ID NO: 78 - DNA, 19 bp, Nicotiana tabacum
  misc_feature 1..19: note = source = /organism="Nicotiana tabacum" /note="Table 2: FK1130-R" /mol_type="unassigned DNA"
  source 1..19: mol_type = genomic DNA
ggcccaatggataaggcgt

SEQ ID NO: 79 - DNA, 21 bp, Nicotiana tabacum
  misc_feature 1..21: note = source = /organism="Nicotiana tabacum" /note="Table 2: FK1131-F" /mol_type="unassigned DNA"
  source 1..21: mol_type = genomic DNA
cagtgcagctgcttgagaaga

SEQ ID NO: 80 - DNA, 21 bp, Nicotiana tabacum
  misc_feature 1..21: note = source = /organism="Nicotiana tabacum" /note="Table 2: FK1132-R" /mol_type="unassigned DNA"
  source 1..21: mol_type = genomic DNA
gtcttcccccttaaccactcg

SEQ ID NO: 81 - DNA, 20 bp, Nicotiana tabacum
  misc_feature 1..20: note = source = /organism="Nicotiana tabacum" /note="Table 2: FK1133-F" /mol_type="unassigned DNA"
  source 1..20: mol_type = genomic DNA
ggtttgcccgagtggttaag

SEQ ID NO: 82 - DNA, 21 bp, Nicotiana tabacum
  misc_feature 1..21: note = source = /organism="Nicotiana tabacum" /note="Table 2: FK1134-R" /mol_type="unassigned DNA"
  source 1..21: mol_type = genomic DNA
gacaaggtgcagcttctttga

SEQ ID NO: 83 - DNA, 25 bp, Nicotiana tabacum
  misc_feature 1..25: note = source = /organism="Nicotiana tabacum" /note="Table 2: FK1135-F" /mol_type="unassigned DNA"
  source 1..25: mol_type = genomic DNA
ctctgaacaagaagaaggattaagg

SEQ ID NO: 84 - DNA, 20 bp, Nicotiana tabacum
  misc_feature 1..20: note = source = /organism="Nicotiana tabacum" /note="Table 2: FK1136-R" /mol_type="unassigned DNA"
  source 1..20: mol_type = genomic DNA
ccttagaccactcggccatc

SEQ ID NO: 85 - DNA, 24 bp, Nicotiana tabacum
  misc_feature 1..24: note = source = /organism="Nicotiana tabacum" /note="Table 2: FK1137-F" /mol_type="unassigned DNA"
  source 1..24: mol_type = genomic DNA
gacttctacggataaagactctga

SEQ ID NO: 86 - DNA, 20 bp, Nicotiana tabacum
  misc_feature 1..20: note = source = /organism="Nicotiana tabacum" /note="Table 2: FK1138-R" /mol_type="unassigned DNA"
  source 1..20: mol_type = genomic DNA
tctaaggcgccagactcaag

SEQ ID NO: 87 - DNA, 21 bp, Nicotiana tabacum
  misc_feature 1..21: note = source = /organism="Nicotiana tabacum" /note="Table 2: FK1139-F" /mol_type="unassigned DNA"
  source 1..21: mol_type = genomic DNA
gcctcctgctgcttaaactct

SEQ ID NO: 88 - DNA, 20 bp, Nicotiana tabacum
  misc_feature 1..20: note = source = /organism="Nicotiana tabacum" /note="Table 2: FK1140-R" /mol_type="unassigned DNA"
  source 1..20: mol_type = genomic DNA
gtaagcgggaggtcttgagt

SEQ ID NO: 89 - DNA, 21 bp, Nicotiana tabacum
  misc_feature 1..21: note = source = /organism="Nicotiana tabacum" /note="Table 2: FK1141-F" /mol_type="unassigned DNA"
  source 1..21: mol_type = genomic DNA
gctccaaaggcaaaagcaaac

SEQ ID NO: 90 - DNA, 20 bp, Nicotiana tabacum
  misc_feature 1..20: note = source = /organism="Nicotiana tabacum" /note="Table 2: FK1142-R" /mol_type="unassigned DNA"
  source 1..20: mol_type = genomic DNA
aacgggtgctctaaccaact

SEQ ID NO: 91 - DNA, 20 bp, Nicotiana tabacum
  misc_feature 1..20: note = source = /organism="Nicotiana tabacum" /note="Table 2: FK1143-F" /mol_type="unassigned DNA"
  source 1..20: mol_type = genomic DNA
gctagcgcgtaggtctcata

SEQ ID NO: 92 - DNA, 20 bp, Nicotiana tabacum
  misc_feature 1..20: note = source = /organism="Nicotiana tabacum" /note="Table 2: FK1144-R" /mol_type="unassigned DNA"
  source 1..20: mol_type = genomic DNA
gaagcaaagctgccgagatg

SEQ ID NO: 93 - DNA, 20 bp, Nicotiana tabacum
  misc_feature 1..20: note = source = /organism="Nicotiana tabacum" /note="Table 2: FK1143-F" /mol_type="unassigned DNA"
  source 1..20: mol_type = genomic DNA
gctagcgcgtaggtctcata

SEQ ID NO: 94 - DNA, 20 bp, Nicotiana tabacum
  misc_feature 1..20: note = source = /organism="Nicotiana tabacum" /note="Table 2: FK1145-R" /mol_type="unassigned DNA"
  source 1..20: mol_type = genomic DNA
ttctccaccgtccatgcaat

SEQ ID NO: 95 - DNA, 20 bp, Nicotiana tabacum
  misc_feature 1..20: note = source = /organism="Nicotiana tabacum" /note="Table 2: FK1146-F" /mol_type="unassigned DNA"
  source 1..20: mol_type = genomic DNA
cgctcgctagagaggaccat

SEQ ID NO: 96 - DNA, 20 bp, Nicotiana tabacum
  misc_feature 1..20: note = source = /organism="Nicotiana tabacum" /note="Table 2: FK1147-R" /mol_type="unassigned DNA"
  source 1..20: mol_type = genomic DNA
gacctacgcgctagccaact

SEQ ID NO: 97 - DNA, 23 bp, Nicotiana tabacum
  misc_feature 1..23: note = source = /organism="Nicotiana tabacum" /note="Table 2: FK1148-F" /mol_type="unassigned DNA"
  source 1..23: mol_type = genomic DNA
ctgaaactgaatcttgcctggag

SEQ ID NO: 98 - DNA, 22 bp, Nicotiana tabacum
  misc_feature 1..22: note = source = /organism="Nicotiana tabacum" /note="Table 2: FK1149-R" /mol_type="unassigned DNA"
  source 1..22: mol_type = genomic DNA
ggactctgaatccagtaacccg

SEQ ID NO: 99 - DNA, 20 bp, Nicotiana tabacum
  misc_feature 1..20: note = source = /organism="Nicotiana tabacum" /note="Table 2: FK1152-F" /mol_type="unassigned DNA"
  source 1..20: mol_type = genomic DNA
actttcatcagccgttttga

SEQ ID NO: 100 - DNA, 22 bp, Nicotiana tabacum
  misc_feature 1..22: note = source = /organism="Nicotiana tabacum" /note="Table 2: FK1153-R" /mol_type="unassigned DNA"
  source 1..22: mol_type = genomic DNA
acgattggttgaatatcatcag

SEQ ID NO: 101 - DNA, 84 bp, Nicotiana tabacum
  misc_feature 1..84: note = source = /organism="Nicotiana tabacum" /note="Fig 5: tRNAmet" /mol_type="unassigned DNA"
  source 1..84: mol_type = genomic DNA
tgaattatcagagtggcgcagcggaagcgtggtgggcccataacccacaggtcccaggatcgaaacctggctctgatatctaga

SEQ ID NO: 102 - DNA, 83 bp, Nicotiana tabacum
  misc_feature 1..83: note = source = /organism="Nicotiana tabacum" /note="Fig 5: tRNAgly" /mol_type="unassigned DNA"
  source 1..83: mol_type = genomic DNA
tgaattgcaccagtggtctagtggcatgatagtaccctgccacggtacagacccgggttcaattcccggctggtgcatctaga

SEQ ID NO: 103 - DNA, 85 bp, Nicotiana tabacum
  misc_feature 1..85: note = source = /organism="Nicotiana tabacum" /note="Fig 5: tRNAIle" /mol_type="unassigned DNA"
  source 1..85: mol_type = genomic DNA
tgaattgctcccgtagctcagttggttagagcgttggtcttatgagccgaaggtcgcgggttcgagccccgccggaagctctaga

SEQ ID NO: 104 - DNA, 71 bp, Nicotiana tabacum
  misc_feature 1..71: note = source = /organism="Nicotiana tabacum" /note="Fig 5: tRNAmet D-loop" /mol_type="unassigned DNA"
  source 1..71: mol_type = genomic DNA
tgaattatcagagtggtggtgggcccataacccacaggtcccaggatcgaaacctggctctgatatctaga

SEQ ID NO: 105 - DNA, 56 bp, Nicotiana tabacum
  misc_feature 1..56: note = source = /organism="Nicotiana tabacum" /note="Fig 5: tRNAmet DA-loop" /mol_type="unassigned DNA"
  source 1..56: mol_type = genomic DNA
tgaattatcagagtggtggcaggtcccaggatcgaaacctggctctgatatctaga

SEQ ID NO: 106 - DNA, 56 bp, Nicotiana tabacum
  misc_feature 1..56: note = source = /organism="Nicotiana tabacum" /note="Fig 5: tRNAmet DT-loop" /mol_type="unassigned DNA"
  source 1..56: mol_type = genomic DNA
tgaattatcagagtggtggtgggcccataacccacaggtccgctctgatatctaga

SEQ ID NO: 107 - DNA, 54 bp, Nicotiana tabacum
  misc_feature 1..54: note = source = /organism="Nicotiana tabacum" /note="Fig 5: tRNAmet AT-loop" /mol_type="unassigned DNA"
  source 1..54: mol_type = genomic DNA
tgaattatcagagtggcgcagcggaagcgtggcaggtccgctctgatatctaga

SEQ ID NO: 108 - RNA, 72 nt, Nicotiana tabacum
  misc_feature 1..72: note = source = /organism="Nicotiana tabacum" /note="Fig 8: tRNAmet" /mol_type="unassigned RNA"
  source 1..72: mol_type = genomic RNA
atcagagtggcgcagcggaagcgtggtgggcccataacccacaggtcccaggatcgaaacctggctctgata

SEQ ID NO: 109 - RNA, 70 nt, Nicotiana tabacum
  misc_feature 1..70: note = source = /organism="Nicotiana tabacum" /note="Fig 8: tRNAgly" /mol_type="unassigned RNA"
  source 1..70: mol_type = genomic RNA
gcaccagtggtctagtggcatgatagtaccctgccacggtacagacccgggttcaattcccggctggtgc

SEQ ID NO: 110 - RNA, 73 nt, Nicotiana tabacum
  misc_feature 1..73: note = source = /organism="Nicotiana tabacum" /note="Fig 8: tRNA Ile" /mol_type="unassigned RNA"
  source 1..73: mol_type = genomic RNA
gctcccgtagctcagttggttagagcgttggtcttatgagccgaaggtcgcgggttcgagccccgccggaagc